European Patent Specification EP 3 661 528 B1, published January 15, 2025. Title: REAGENTS FOR EXPANDING CELLS EXPRESSING RECOMBINANT RECEPTORS. Applicant: Juno Therapeutics, Inc. HAUSKINS, Collin HUSSELL, Scott SIERRA, Catherine WORKS, Melissa. Application Not Yet Assigned. The sequence listing filed with the application follows.

SEQUENCE LISTING (154 sequences)

SEQ ID NO: 1 - protein, 54 aa, Homo sapiens
MLQMAGQCSQNEYFDSLLHACIPCQLRCSSNTPPLTCQRYCNASVTNSVKGTNA

SEQ ID NO: 2 - protein, 232 aa, Homo sapiens
EPKSCDKTHTCPPCPAPELLGGPSVFLFPPKPKDTLMISRTPEVTCVVVDVSHEDPEVKFNWYVDGVEVHNAKTKPREEQYNSTYRVVSVLTVLHQDWLNGKEYKCKVSNKALPAPIEKTISKAKGQPREPQVYTLPPSREEMTKNQVSLTCLVKGFYPSDIAVEWESNGQPENNYKTTPPVLDSDGSFFLYSKLTVDKSRWQQGNVFSCSVMHEALHNHYTQKSLSLSPGK

SEQ ID NO: 3 - protein, 15 aa, Artificial Sequence
  AviTag
GLNDIFEAQKIEWHE

SEQ ID NO: 4 - protein, 26 aa, Artificial Sequence
  Calmodulin Tag
KRRWKKNFIAVSAANRFKKISSSGAL

SEQ ID NO: 5 - protein, 6 aa, Artificial Sequence
  Polyglutamine tag
EEEEEE

SEQ ID NO: 6 - protein, 8 aa, Artificial Sequence
  Flag-tag
DYKDDDDK

SEQ ID NO: 7 - protein, 9 aa, Artificial Sequence
  HA-tag
YPYDVPDYA

SEQ ID NO: 8 - protein, 10 aa, Artificial Sequence
  Myc-tag
EQKLISEEDL

SEQ ID NO: 9 - protein, 8 aa, Artificial Sequence
  STREP-TAG(r) I streptavidin-binding peptide sequence
WRHPQFGG

SEQ ID NO: 10 - protein, 8 aa, Artificial Sequence
  STREP-TAG(r) II streptavidin-binding peptide sequence
WSHPQFEK

SEQ ID NO: 11 - protein, 4 aa, Artificial Sequence
  Streptavidin Binding peptide
  misc_feature (3)..(3): X is selected from glutamine, asparagine and methionine
  misc_feature (4)..(4): X is no amino acid
HPXX

SEQ ID NO: 12 - protein, 4 aa, Artificial Sequence
  Streptavidin Binding peptide
HPQF

SEQ ID NO: 13 - protein, 8 aa, Artificial Sequence
  Streptavidin Binding peptide
  misc_feature (1)..(1): Xaa = is Trp, Lys or Arg
  misc_feature (2)..(2): Xaa = any amino acid
  misc_feature (7)..(7): Xaa =  Gly or Glu
  misc_feature (8)..(8): Xaa =  Gly, Lys or Arg
XXHPQFXX

SEQ ID NO: 14 - protein, 8 aa, Artificial Sequence
  Streptavidin Binding peptide
  misc_feature (2)..(2): Xaa is any amino acid
  misc_feature (7)..(7): Xaa is Gly or Glu
  misc_feature (8)..(8): Xaa is Gly, Lys or Arg
WXHPQFXX

SEQ ID NO: 15 - protein, 17 aa, Artificial Sequence
  Streptavidin Binding peptide
  misc_feature (9)..(9): Xaa is any amino
  REPEAT (9)..(9): n = 8 or 12
WSHPQFEKXWSHPQFEK

SEQ ID NO: 16 - protein, 21 aa, Artificial Sequence
  Streptavidin Binding peptide
  misc_feature: Streptavidin Binding peptide
  REPEAT (9)..(12): N = 2 OR 3
WSHPQFEKGGGSNWSHPQFEK

SEQ ID NO: 17 - protein, 30 aa, Artificial Sequence
  Streptavidin Binding peptide
SAWSHPQFEKGGGSGGGSGGGSWSHPQFEK

SEQ ID NO: 18 - protein, 30 aa, Artificial Sequence
  Streptavidin Binding peptide
SAWSHPQFEKGGGSGGGSGGSAWSHPQFEK

SEQ ID NO: 19 - protein, 28 aa, Artificial Sequence
  Streptavidin Binding peptide
WSHPQFEKGGGSGGGSGGGSWSHPQFEK

SEQ ID NO: 20 - protein, 24 aa, Artificial Sequence
  Streptavidin Binding peptide
WSHPQFEKGGGSGGGSWSHPQFEK

SEQ ID NO: 21 - protein, 28 aa, Artificial Sequence
  Streptavidin Binding peptide
WSHPQFEKGGGSGGGSGGSAWSHPQFEK

SEQ ID NO: 22 - protein, 159 aa, Streptomyces avidinii
  misc_feature: Wild type Streptavidin Sequence (Streptavidin- Species: Streptomyces avidinii - UniProt No. P22629
DPSKDSKAQVSAAEAGITGTWYNQLGSTFIVTAGADGALTGTYESAVGNAESRYVLTGRYDSAPATDGSGTALGWTVAWKNNYRNAHSATTWSGQYVGGAEARINTQWLLTSGTTEANAWKSTLVGHDTFTKVKPSAASIDAAKKAGVNNGNPLDAVQQ

SEQ ID NO: 23 - protein, 126 aa, Artificial Sequence
  mutein streptavidin designated Strep-tactin(r)
EAGITGTWYNQLGSTFIVTAGADGALTGTYVTARGNAESRYVLTGRYDSAPATDGSGTALGWTVAWKNNYRNAHSATTWSGQYVGGAEARINTQWLLTSGTTEANAWKSTLVGHDTFTKVKPSAAS

SEQ ID NO: 24 - protein, 340 aa, Artificial Sequence
  Sleeping Beauty Transposase
MGKSKEISQDLRKKIVDLHKSGSSLGAISKRLKVPRSSVQTIVRKYKHHGTTQPSYRSGRRRVLSPRDERTLVRKVQINPRTTAKDLVKMLEETGTKVSISTVKRVLYRHNLKGRSARKKPLLQNRHKKARLRFATAHGDKDRTFWRNVLWSDETKIELFGHNDHRYVWRKKGEACKPKNTIPTVKHGGGSIMLWCGFAAGGTGALHKIDGIMRKENYVDILKQHLKTSVRKLKLGRKWVFQMDNDPKHTSKVVAKWLKDNKVKVLEWPSQSPDLNPIENLWAELKKRVRARRPTNLTQLHQLCQEEWAKIHPTYCGKLVEGYPKRLTQVKQFKGNATKY

SEQ ID NO: 25 - DNA, 1083 bp, Artificial Sequence
  Sleeping Beauty Transpose
atgggaaaatcaaaagaaatcagccaagacctcagaaaaaaaattgtagacctccacaagtctggttcatccttgggagcaatttccaaacgcctgaaagtaccacgttcatctgtacaatctggttcatccttgggagcaatttccaaacgcctgaaagtaccacgttcatctgtacaaacaatagtacgcaagtataaacaccatgggaccacgcagccgtcataccgctcaggaaggagacgcgttctgtctcctagagatgaacgtactttggtgcgaaaagtgcaaatcaatcccagaacaacagcaaaggaccttgtgaagatgctggaggaaacaggtacaaaagtatctatatccacagtaaaacgagtcctatatcgacataacctgaaaggccgctcagcaaggaagaagccactgctccaaaaccgacataagaaagccagactacggtttgcaactgcacatggggacaaagatcgtactttttggagaaatgtcctctggtctgatgaaacaaaaatagaactgtttggccataatgaccatcgttatgtttggaggaagaagggggaggcttgcaagccgaagaacaccatcccaaccgtgaagcacgggggtggcagcatcatgttgtgggggtgctttgctgcaggagggactggtgcacttcacaaaatagatggcatcatgaggaaggaaaattatgtggatatattgaagcaacatctcaagacatgagtcaggaagttaaagcttggtcgcaaatgggtcttccaaatggacaatgaccccaagcatacttccaaagttgtggcaaaatggcttaaggacaacaaagtcaaggtattggagtggccatcacaaagccctgacctcaatcctatagaaaatttgtgggcagaactgaaaaagcgtgtgcgagcaaggaggcctacaaacctgactcagttacaccagctctgtcaggaggaatgggccaaaattcacccaacttattgtgggaagcttgtggaaggctacccgaaacgtttgacccaagttaaacaatttaaaggcaatgctaccaaatactag

SEQ ID NO: 26 - DNA, 352 bp, Artificial Sequence
  Sleeping Beauty inverted repeat sequence
cagttgaagtcggaagtttacatacacttaagttggagtcattaaaactcgtttttcaactactccacaaatttcttgttaacaaacaatagttttggcaagtcagttaggacatctactttgtgcatgacacaagtcatttttccaacaattgtttacagacagattatttcacttataattcactgtatcacaattccagtgggtcagaagtttacatacactaagttgactgtgcctttaaacagcttggaaaattccagaaaatgatgtcatggctttagaagcttctgatagactaattgacatcatttgagtcaattggaggtgtacctgtggatgtatttcaagg

SEQ ID NO: 27 - protein, 5 aa, Artificial Sequence
  Linker sequence
GGGGS

SEQ ID NO: 28 - protein, 231 aa, Artificial Sequence
  Modified Human IgG1 Fc
PKSSDKTHTCPPCPAPEAEGAPSVFLFPPKPKDTLMISRTPEVTCVVVDVSHEDPEVKFNWYVDGVEVHNAKTKPREEQYNSTYRVVSVLTVLHQDWLNGKEYKCKVSNKALPSSIEKTISKAKGQPREPQVYTLPPSRDELTKNQVSLTCLVKGFYPSDIAVEWESNGQPENNYKTTPPVLDSDGSFFLYSKLTVDKSRWQQGNVFSCSVMHEALHNHYTQKSLSLSPGK

SEQ ID NO: 29 - protein, 668 aa, Homo sapiens
  misc_feature: Human CD22 extracellular domain
DSSKWVFEHPETLYAWEGACVWIPCTYRALDGDLESFILFHNPEYNKNTSKFDGTRLYESTKDGKVPSEQKRVQFLGDKNKNCTLSIHPVHLNDSGQLGLRMESKTEKWMERIHLNVSERPFPPHIQLPPEIQESQEVTLTCLLNFSCYGYPIQLQWLLEGVPMRQAAVTSTSLTIKSVFTRSELKFSPQWSHHGKIVTCQLQDADGKFLSNDTVQLNVKHTPKLEIKVTPSDAIVREGDSVTMTCEVSSSNPEYTTVSWLKDGTSLKKQNTFTLNLREVTKDQSGKYCCQVSNDVGPGRSEEVFLQVQYAPEPSTVQILHSPAVEGSQVEFLCMSLANPLPTNYTWYHNGKEMQGRTEEKVHIPKILPWHAGTYSCVAENILGTGQRGPGAELDVQYPPKKVTTVIQNPMPIREGDTVTLSCNYNSSNPSVTRYEWKPHGAWEEPSLGVLKIQNVGWDNTTIACAACNSWCSWASPVALNVQYAPRDVRVRKIKPLSEIHSGNSVSLQCDFSSSHPKEVQFFWEKNGRLLGKESQLNFDSISPEDAGSYSCWVNNSIGQTASKAWTLEVLYAPRRLRVSMSPGDQVMEGKSATLTCESDANPPVSHYTWFDWNNQSLPYHSQKLRLEPVKVQHSGAYWCQGTNSVGKGRSPLSTLTVYYSPETIGRR

SEQ ID NO: 30 - protein, 16 aa, Artificial Sequence
  CD33 Signal peptide
MPLLLLLPLLWAGALA

SEQ ID NO: 31 - protein, 377 aa, Homo sapiens
  misc_feature: Human ROR1 fragment
QETELSVSAELVPTSSWNISSELNKDSYLTLDEPMNNITTSLGQTAELHCKVSGNPPPTIRWFKNDAPVVQEPRRLSFRSTIYGSRLRIRNLDTTDTGYFQCVATNGKEVVSSTGVLFVKFGPPPTASPGYSDEYEEDGFCQPYRGIACARFIGNRTVYMESLHMQGEIENQITAAFTMIGTSSHLSDKCSQFAIPSLCHYAFPYCDETSSVPKPRDLCRDECEILENVLCQTEYIFARSNPMILMRLKLPNCEDLPQPESPEAANCIRIGIPMADPINKNHKCYNSTGVDYRGTVSVTKSGRQCQPWNSQYPHTHTFTALRFPELNGGHSYCRNPGNQKEAPWCFTLDENFKSDLCDIPACDSKDSKEKNKMEILY

SEQ ID NO: 32 - protein, 22 aa, Artificial Sequence
  F2A
VKQTLNFDLLKLAGDVESNPGP

SEQ ID NO: 33 - protein, 613 aa, Artificial Sequence
  ROR1-Fc fusion polypeptide
QETELSVSAELVPTSSWNISSELNKDSYLTLDEPMNNITTSLGQTAELHCKVSGNPPPTIRWFKNDAPVVQEPRRLSFRSTIYGSRLRIRNLDTTDTGYFQCVATNGKEVVSSTGVLFVKFGPPPTASPGYSDEYEEDGFCQPYRGIACARFIGNRTVYMESLHMQGEIENQITAAFTMIGTSSHLSDKCSQFAIPSLCHYAFPYCDETSSVPKPRDLCRDECEILENVLCQTEYIFARSNPMILMRLKLPNCEDLPQPESPEAANCIRIGIPMADPINKNHKCYNSTGVDYRGTVSVTKSGRQCQPWNSQYPHTHTFTALRFPELNGGHSYCRNPGNQKEAPWCFTLDENFKSDLCDIPACDSKDSKEKNKMEILYGGGGSPKSSDKTHTCPPCPAPEAEGAPSVFLFPPKPKDTLMISRTPEVTCVVVDVSHEDPEVKFNWYVDGVEVHNAKTKPREEQYNSTYRVVSVLTVLHQDWLNGKEYKCKVSNKALPSSIEKTISKAKGQPREPQVYTLPPSRDELTKNQVSLTCLVKGFYPSDIAVEWESNGQPENNYKTTPPVLDSDGSFFLYSKLTVDKSRWQQGNVFSCSVMHEALHNHYTQKSLSLSPGK

SEQ ID NO: 34 - protein, 904 aa, Artificial Sequence
  CD22-Fc fusion polypeptide
DSSKWVFEHPETLYAWEGACVWIPCTYRALDGDLESFILFHNPEYNKNTSKFDGTRLYESTKDGKVPSEQKRVQFLGDKNKNCTLSIHPVHLNDSGQLGLRMESKTEKWMERIHLNVSERPFPPHIQLPPEIQESQEVTLTCLLNFSCYGYPIQLQWLLEGVPMRQAAVTSTSLTIKSVFTRSELKFSPQWSHHGKIVTCQLQDADGKFLSNDTVQLNVKHTPKLEIKVTPSDAIVREGDSVTMTCEVSSSNPEYTTVSWLKDGTSLKKQNTFTLNLREVTKDQSGKYCCQVSNDVGPGRSEEVFLQVQYAPEPSTVQILHSPAVEGSQVEFLCMSLANPLPTNYTWYHNGKEMQGRTEEKVHIPKILPWHAGTYSCVAENILGTGQRGPGAELDVQYPPKKVTTVIQNPMPIREGDTVTLSCNYNSSNPSVTRYEWKPHGAWEEPSLGVLKIQNVGWDNTTIACAACNSWCSWASPVALNVQYAPRDVRVRKIKPLSEIHSGNSVSLQCDFSSSHPKEVQFFWEKNGRLLGKESQLNFDSISPEDAGSYSCWVNNSIGQTASKAWTLEVLYAPRRLRVSMSPGDQVMEGKSATLTCESDANPPVSHYTWFDWNNQSLPYHSQKLRLEPVKVQHSGAYWCQGTNSVGKGRSPLSTLTVYYSPETIGRRGGGGSPKSSDKTHTCPPCPAPEAEGAPSVFLFPPKPKDTLMISRTPEVTCVVVDVSHEDPEVKFNWYVDGVEVHNAKTKPREEQYNSTYRVVSVLTVLHQDWLNGKEYKCKVSNKALPSSIEKTISKAKGQPREPQVYTLPPSRDELTKNQVSLTCLVKGFYPSDIAVEWESNGQPENNYKTTPPVLDSDGSFFLYSKLTVDKSRWQQGNVFSCSVMHEALHNHYTQKSLSLSPGK

SEQ ID NO: 35 - protein, 290 aa, Artificial Sequence
  BCMA-Fc fusion polypeptide
MLQMAGQCSQNEYFDSLLHACIPCQLRCSSNTPPLTCQRYCNASVTNSVKGTNAGGGGSPKSSDKTHTCPPCPAPEAEGAPSVFLFPPKPKDTLMISRTPEVTCVVVDVSHEDPEVKFNWYVDGVEVHNAKTKPREEQYNSTYRVVSVLTVLHQDWLNGKEYKCKVSNKALPSSIEKTISKAKGQPREPQVYTLPPSRDELTKNQVSLTCLVKGFYPSDIAVEWESNGQPENNYKTTPPVLDSDGSFFLYSKLTVDKSRWQQGNVFSCSVMHEALHNHYTQKSLSLSPGK

SEQ ID NO: 36 - protein, 122 aa, Artificial Sequence
  SJ25C1 veriable heavy chain
EVKLQQSGAELVRPGSSVKISCKASGYAFSSYWMNWVKQRPGQGLEWIGQIYPGDGDTNYNGKFKGQATLTADKSSSTAYMQLSGLTSEDSAVYFCARKTISSVVDFYFDYWGQGTTVTVSS

SEQ ID NO: 37 - protein, 108 aa, Artificial Sequence
  SJ25C1 variable light chain
DIELTQSPKFMSTSVGDRVSVTCKASQNVGTNVAWYQQKPGQSPKPLIYSATYRNSGVPDRFTGSGSGTDFTLTITNVQSKDLADYFCQQYNRYPYTSGGGTKLEIKR

SEQ ID NO: 38 - protein, 120 aa, Artificial Sequence
  FMC63 variable heavy chain
EVKLQESGPGLVAPSQSLSVTCTVSGVSLPDYGVSWIRQPPRKGLEWLGVIWGSETTYYNSALKSRLTIIKDNSKSQVFLKMNSLQTDDTAIYYCAKHYYYGGSYAMDYWGQGTSVTVSS

SEQ ID NO: 39 - protein, 107 aa, Artificial Sequence
  FMC63 variable light chain
DIQMTQTTSSLSASLGDRVTISCRASQDISKYLNWYQQKPDGTVKLLIYHTSRLHSGVPSRFSGSGSGTDYSLTISNLEQEDIATYFCQQGNTLPYTFGGGTKLEIT

SEQ ID NO: 40 - protein, 5 aa, Artificial Sequence
  SJ25C1 HC-CDR1
SYWMN

SEQ ID NO: 41 - protein, 17 aa, Artificial Sequence
  SJ25C1 HC-CDR2
QIYPGDGDTNYNGKFKG

SEQ ID NO: 42 - protein, 13 aa, Artificial Sequence
  SJ25C1 HC-CDR3
KTISSVVDFYFDY

SEQ ID NO: 43 - protein, 11 aa, Artificial Sequence
  SJ25C1 LC-CDR1
KASQNVGTNVA

SEQ ID NO: 44 - protein, 7 aa, Artificial Sequence
  SJ25C1 LC-CDR2
SATYRNS

SEQ ID NO: 45 - protein, 9 aa, Artificial Sequence
  SJ25C1 LC-CDR3
QQYNRYPYT

SEQ ID NO: 46 - protein, 5 aa, Artificial Sequence
  FMC63 HC-CDR1
DYGVS

SEQ ID NO: 47 - protein, 16 aa, Artificial Sequence
  FMC63 HC-CDR2
VIWGSETTYYNSALKS

SEQ ID NO: 48 - protein, 12 aa, Artificial Sequence
  FMC63 HC-CDR3
HYYYGGSYAMDY

SEQ ID NO: 49 - protein, 11 aa, Artificial Sequence
  FMC63 LC-CDR1
RASQDISKYLN

SEQ ID NO: 50 - protein, 7 aa, Artificial Sequence
  FMC63 LC-CDR2
HTSRLHS

SEQ ID NO: 51 - protein, 9 aa, Artificial Sequence
  FMC63 LC-CDR3
QQGNTLPYT

SEQ ID NO: 52 - protein, 122 aa, Artificial Sequence
  anti-ID VH
QVQLQQPGSELVRPGGSVKLSCKASDYTFTSYWMHWVRQRPGQGLEWIGNIYPGSGGTNYDEKFKRKATLTVDTSSSTAYMQLRSLTSEDSAVYYCTREVTTVAYYYSMDYWGQGTSVTVSS

SEQ ID NO: 53 - protein, 13 aa, Artificial Sequence
  anti-ID HC-CDR3
EVTTVAYYYSMDY

SEQ ID NO: 54 - protein, 14 aa, Artificial Sequence
  anti-ID HC-CDR3
TREVTTVAYYYSMD

SEQ ID NO: 55 - protein, 5 aa, Artificial Sequence
  anti-ID HC-CDR1
SYWMH

SEQ ID NO: 56 - protein, 7 aa, Artificial Sequence
  anti-ID HC-CDR1
DYTFTSY

SEQ ID NO: 57 - protein, 10 aa, Artificial Sequence
  anti-ID HC-CDR1
DYTFTSYWMH

SEQ ID NO: 58 - protein, 6 aa, Artificial Sequence
  anti-ID HC-CDR1
TSYWMH

SEQ ID NO: 59 - protein, 17 aa, Artificial Sequence
  anti-ID HC-CDR2
NIYPGSGGTNYDEKFKR

SEQ ID NO: 60 - protein, 6 aa, Artificial Sequence
  anti-ID HC-CDR2
YPGSGG

SEQ ID NO: 61 - protein, 10 aa, Artificial Sequence
  anti-ID HC-CDR2
NIYPGSGGTN

SEQ ID NO: 62 - protein, 13 aa, Artificial Sequence
  anti-ID HC-CDR2
WIGNIYPGSGGTN

SEQ ID NO: 63 - protein, 107 aa, Artificial Sequence
  anti-ID VL
DIQMTQTTSSLSASLGDRVTISCRASQDISNYLNWYQQKPDGTVKLLIYYTSRLHSGVPSRFSGSGSGTDYSLTISNLEQEDIATYFCQQGKTVPFTFGSGTKLEIK

SEQ ID NO: 64 - protein, 9 aa, Artificial Sequence
  anti-ID LC-CDR3
QQGKTVPFT

SEQ ID NO: 65 - protein, 8 aa, Artificial Sequence
  anti-ID LC-CDR3
QQGKTVPF

SEQ ID NO: 66 - protein, 11 aa, Artificial Sequence
  anti-ID LC-CDR1
RASQDISNYLN

SEQ ID NO: 67 - protein, 7 aa, Artificial Sequence
  anti-ID LC-CDR1
SNYLNWY

SEQ ID NO: 68 - protein, 7 aa, Artificial Sequence
  anti-ID LC-CDR2
YTSRLHS

SEQ ID NO: 69 - protein, 10 aa, Artificial Sequence
  anti-ID LC-CDR2
LLIYYTSRLH

SEQ ID NO: 70 - protein, 4 aa, Artificial Sequence
  linker sequence
GGGS

SEQ ID NO: 71 - protein, 15 aa, Artificial Sequence
  linker sequence
GGGGSGGGGSGGGGS

SEQ ID NO: 72 - protein, 18 aa, Artificial Sequence
  Linker
GSTSGSGKPGSGEGSTKG

SEQ ID NO: 73 - protein, 122 aa, Artificial Sequence
  anti-ID B-1 VH
EVQLQQSGPELVKPGASVKMSCKASGYTFTDYYMKWVKQCHGKSLEWIGDINPNNGGTDYNQNFKGKATLTVDKSSSTAYMQLNSLTSEDSAVYYCAREGNNYGSRDAMDYWGQGTSVTVSS

SEQ ID NO: 74 - protein, 115 aa, Artificial Sequence
  anti-ID B-2 VH
QVQLQQPGAELVRPGASVKLSCKTSGYSFTRYWMNWVKQRPGQGLEWIGMIHPSDSETRLNQKFKDKATLTVDNSSSTAYMQLSSPTSEDSAVYYCASIYYEEAWGQGTLVTVSA

SEQ ID NO: 75 - protein, 13 aa, Artificial Sequence
  anti-ID B-1 HC-CDR3
EGNNYGSRDAMDY

SEQ ID NO: 76 - protein, 6 aa, Artificial Sequence
  anti-ID B-2 HC-CDR3
IYYEEA

SEQ ID NO: 77 - protein, 14 aa, Artificial Sequence
  anti-ID B-1 HC-CDR3
AREGNNYGSRDAMD

SEQ ID NO: 78 - protein, 7 aa, Artificial Sequence
  anti-ID B-2 HC-CDR3
ASIYYEE

SEQ ID NO: 79 - protein, 5 aa, Artificial Sequence
  anti-ID B-1 HC-CDR1
DYYMK

SEQ ID NO: 80 - protein, 5 aa, Artificial Sequence
  anti-ID B-2 HC-CDR1
RYWMN

SEQ ID NO: 81 - protein, 7 aa, Artificial Sequence
  anti-ID B-1 HC-CDR1
GYTFTDY

SEQ ID NO: 82 - protein, 10 aa, Artificial Sequence
  anti-ID B-1 HC-CDR1
GYTFTDYYMK

SEQ ID NO: 83 - protein, 6 aa, Artificial Sequence
  anti-ID B-1 HC-CDR1
TDYYMK

SEQ ID NO: 84 - protein, 7 aa, Artificial Sequence
  anti-ID B-2 HC-CDR1
GYSFTRY

SEQ ID NO: 85 - protein, 10 aa, Artificial Sequence
  anti-ID B-2 HC-CDR1
GYSFTRYWMN

SEQ ID NO: 86 - protein, 6 aa, Artificial Sequence
  anti-ID B-2 HC-CDR1
TRYWMN

SEQ ID NO: 87 - protein, 17 aa, Artificial Sequence
  anti-ID B-1 HC-CDR2
DINPNNGGTDYNQNFKG

SEQ ID NO: 88 - protein, 17 aa, Artificial Sequence
  anti-ID B-2 HC-CDR2
MIHPSDSETRLNQKFKD

SEQ ID NO: 89 - protein, 6 aa, Artificial Sequence
  anti-ID B-1 HC-CDR2
NPNNGG

SEQ ID NO: 90 - protein, 10 aa, Artificial Sequence
  anti-ID B-1 HC-CDR2
DINPNNGGTD

SEQ ID NO: 91 - protein, 13 aa, Artificial Sequence
  anti-ID B-1 HC-CDR2
WIGDINPNNGGTD

SEQ ID NO: 92 - protein, 6 aa, Artificial Sequence
  anti-ID B-2 HC-CDR2
HPSDSE

SEQ ID NO: 93 - protein, 10 aa, Artificial Sequence
  anti-ID B-2 HC-CDR2
MIHPSDSETR

SEQ ID NO: 94 - protein, 13 aa, Artificial Sequence
  anti-ID B-2 HC-CDR2
WIGMIHPSDSETR

SEQ ID NO: 95 - protein, 10 aa, Artificial Sequence
  HC-CDR1 Consensus
  VARIANT (3)..(3): X = T or S
  VARIANT (5)..(5): X = T or S
  VARIANT (6)..(6): X = D or R
  VARIANT (8)..(8): X = Y or W
  VARIANT (10)..(10): X = K or N
GYXFXXYXMX

SEQ ID NO: 96 - protein, 20 aa, Artificial Sequence
  HC-CDR2 Consensus
  VARIANT (4)..(4): X = D or M
  VARIANT (6)..(6): X = N or H
  VARIANT (8)..(8): X = N or S
  VARIANT (9)..(9): X = N or D
  VARIANT (10)..(10): X = G or S
  VARIANT (11)..(11): X = G or E
  VARIANT (13)..(13): X = D or R
  VARIANT (14)..(14): X = Y or L
  VARIANT (17)..(17): X = N or K
  VARIANT (20)..(20): X = G or D
WIGXIXPXXXXTXXNQXFKX

SEQ ID NO: 97 - protein, 15 aa, Artificial Sequence
  HC-CDR3 Consensus
  VARIANT (2)..(2): X=R or S
  VARIANT (3)..(3): X=E or I
  VARIANT (4)..(4): X=G or Y
  VARIANT (5)..(5): X=N or Y
  VARIANT (6)..(6): X=N or E
  VARIANT (7)..(7): X=Y or null
  VARIANT (8)..(8): X=G or null
  VARIANT (9)..(9): X=S or null
  VARIANT (10)..(10): X=R or null
  VARIANT (11)..(11): X=D or null
  VARIANT (12)..(12): X=A or null
  VARIANT (13)..(13): X=M or null
  VARIANT (14)..(14): X=D or E
  VARIANT (15)..(15): X=Y or A
AXXXXXXXXXXXXXX

SEQ ID NO: 98 - protein, 106 aa, Artificial Sequence
  anti-ID B-1 VL
QIVLTQSPALMSASPGEKVTMTCSASSGVIYMYWYQQKPRSSPKPWIYLTSNLASGVPARFSGSGSGTSYSLTISSMEAEDAATYYCQQWSSNPLTFGAGTKLELK

SEQ ID NO: 99 - protein, 107 aa, Artificial Sequence
  anti-ID B-2 VL
DIQMTQSPASLSASVGETVTITCRASGNIHNYLAWYQQKQGKSPQLLVYNAKTLADSVPSRFSGSGSGTQYSLKINSLQPEDFGSYYCQHFWSTPYTFGGGTKLEIK

SEQ ID NO: 100 - protein, 9 aa, Artificial Sequence
  anti-ID B-1 LC-CDR3
QQWSSNPLT

SEQ ID NO: 101 - protein, 8 aa, Artificial Sequence
  anti-ID B-1 LC-CDR3
QQWSSNPL

SEQ ID NO: 102 - protein, 9 aa, Artificial Sequence
  anti-ID B-2 LC-CDR3
QHFWSTPYT

SEQ ID NO: 103 - protein, 8 aa, Artificial Sequence
  anti-ID B-2 LC-CDR3
QHFWSTPY

SEQ ID NO: 104 - protein, 10 aa, Artificial Sequence
  anti-ID B-1 LC-CDR1
SASSGVIYMY

SEQ ID NO: 105 - protein, 11 aa, Artificial Sequence
  anti-ID B-2 LC-CDR1
RASGNIHNYLA

SEQ ID NO: 106 - protein, 6 aa, Artificial Sequence
  anti-ID B-1 LC-CDR1
IYMYWY

SEQ ID NO: 107 - protein, 7 aa, Artificial Sequence
  anti-ID B-2 LC-CDR1
HNYLAWY

SEQ ID NO: 108 - protein, 7 aa, Artificial Sequence
  anti-ID B-1 LC-CDR2
LTSNLAS

SEQ ID NO: 109 - protein, 7 aa, Artificial Sequence
  anti-ID B-2 LC-CDR2
NAKTLAD

SEQ ID NO: 110 - protein, 10 aa, Artificial Sequence
  anti-ID B-1 LC-CDR2
PWIYLTSNLA

SEQ ID NO: 111 - protein, 10 aa, Artificial Sequence
  anti-ID B-2 LC-CDR2
LLVYNAKTLA

SEQ ID NO: 112 - protein, 13 aa, Artificial Sequence
  LC-CDR1 Consensus
  VARIANT (1)..(1): X= S or R
  VARIANT (3)..(3): X= S or R
  VARIANT (4)..(4): X= S or G
  VARIANT (5)..(5): X= G or N
  VARIANT (6)..(6): X= V or I
  VARIANT (7)..(7): X= I or H
  VARIANT (8)..(8): X= N or null
  VARIANT (10)..(10): X= M or L
  VARIANT (11)..(11): X= Y or A
XAXXXXXXYXXWY

SEQ ID NO: 113 - protein, 11 aa, Artificial Sequence
  LC-CDR2 Consensus
  VARIANT (1)..(1): X= P or L
  VARIANT (2)..(2): X= W or L
  VARIANT (3)..(3): X= I or V
  VARIANT (5)..(5): X= L or N
  VARIANT (6)..(6): X= T or A
  VARIANT (7)..(7): X= S or K
  VARIANT (8)..(8): X= N or T
  VARIANT (11)..(11): X= S or D
XXXYXXXXLAX

SEQ ID NO: 114 - protein, 9 aa, Artificial Sequence
  LC-CDR3 Consensus
  VARIANT (2)..(2): X= Q or H
  VARIANT (3)..(3): X= W or F
  VARIANT (4)..(4): X= S or W
  VARIANT (5)..(5): X= S or W
  VARIANT (6)..(6): X= N or T
  VARIANT (8)..(8): X= L or Y
QXXXXXPXT

SEQ ID NO: 115 - protein, 324 aa, Artificial Sequence
  anti-ID CH
AKTTPPSVYPLAPGSAAQTNSMVTLGCLVKGYFPEPVTVTWNSGSLSSGVHTFPAVLQSDLYTLSSSVTVPSSTWPSETVTCNVAHPASSTKVDKKIVPRDCGCKPCICTVPEVSSVFIFPPKPKDVLTITLTPKVTCVVVDISKDDPEVQFSWFVDDVEVHTAQTQPREEQFNSTFRSVSELPIMHQDWLNGKEFKCRVNSAAFPAPIEKTISKTKGRPKAPQVYTIPPPKEQMAKDKVSLTCMITDFFPEDITVEWQWNGQPAENYKNTQPIMDTDGSYFVYSKLNVQKSNWEAGNTFTCSVLHEGLHNHHTEKSLSHSPGK

SEQ ID NO: 116 - protein, 446 aa, Artificial Sequence
  anti-ID heavy chain
QVQLQQPGSELVRPGGSVKLSCKASDYTFTSYWMHWVRQRPGQGLEWIGNIYPGSGGTNYDEKFKRKATLTVDTSSSTAYMQLRSLTSEDSAVYYCTREVTTVAYYYSMDYWGQGTSVTVSSAKTTPPSVYPLAPGSAAQTNSMVTLGCLVKGYFPEPVTVTWNSGSLSSGVHTFPAVLQSDLYTLSSSVTVPSSTWPSETVTCNVAHPASSTKVDKKIVPRDCGCKPCICTVPEVSSVFIFPPKPKDVLTITLTPKVTCVVVDISKDDPEVQFSWFVDDVEVHTAQTQPREEQFNSTFRSVSELPIMHQDWLNGKEFKCRVNSAAFPAPIEKTISKTKGRPKAPQVYTIPPPKEQMAKDKVSLTCMITDFFPEDITVEWQWNGQPAENYKNTQPIMDTDGSYFVYSKLNVQKSNWEAGNTFTCSVLHEGLHNHHTEKSLSHSPGK

SEQ ID NO: 117 - protein, 19 aa, Artificial Sequence
  anti-ID HC signal sequence
MGWSSIILFLVATASGVHS

SEQ ID NO: 118 - protein, 107 aa, Artificial Sequence
  anti-ID CL
RADAAPTVSIFPPSSEQLTSGGASVVCFLNNFYPKDINVKWKIDGSERQNGVLNSWTDQDSKDSTYSMSSTLTLTKDEYERHNNYTCEATHKTSTSPIVKSFNRNEC

SEQ ID NO: 119 - protein, 214 aa, Artificial Sequence
  anti-ID light chain
DIQMTQTTSSLSASLGDRVTISCRASQDISNYLNWYQQKPDGTVKLLIYYTSRLHSGVPSRFSGSGSGTDYSLTISNLEQEDIATYFCQQGKTVPFTFGSGTKLEIKRADAAPTVSIFPPSSEQLTSGGASVVCFLNNFYPKDINVKWKIDGSERQNGVLNSWTDQDSKDSTYSMSSTLTLTKDEYERHNNYTCEATHKTSTSPIVKSFNRNEC

SEQ ID NO: 120 - protein, 20 aa, Artificial Sequence
  anti-ID LC signal sequence
MMSSAQFLGLLLLCFQGTRC

SEQ ID NO: 121 - protein, 330 aa, Artificial Sequence
  anti-ID B-1 CH
AKTTAPSVYPLAPVCGDTTGSSVTLGCLVKGYFPEPVTLTWNSGSLSSGVHTFPAVLQSDLYTLSSSVTVTSSTWPSQSITCNVAHPASSTKVDKKIEPRGPTIKPCPPCKCPAPNLLGGPSVFIFPPKIKDVLMISLSPIVTCVVVDVSEDDPDVQISWFVNNVEVHTAQTQTHREDYNSTLRVVSALPIQHQDWMSGKEFKCKVNNKDLPAPIERTISKPKGSVRAPQVYVLPPPEEEMTKKQVTLTCMVTDFMPEDIYVEWTNNGKTELNYKNTEPVLDSDGSYFMYSKLRVEKKNWVERNSYSCSVVHEGLHNHHTTKSFSRTPGK

SEQ ID NO: 122 - protein, 452 aa, Artificial Sequence
  anti-ID B-1 heavy chain
EVQLQQSGPELVKPGASVKMSCKASGYTFTDYYMKWVKQCHGKSLEWIGDINPNNGGTDYNQNFKGKATLTVDKSSSTAYMQLNSLTSEDSAVYYCAREGNNYGSRDAMDYWGQGTSVTVSSAKTTAPSVYPLAPVCGDTTGSSVTLGCLVKGYFPEPVTLTWNSGSLSSGVHTFPAVLQSDLYTLSSSVTVTSSTWPSQSITCNVAHPASSTKVDKKIEPRGPTIKPCPPCKCPAPNLLGGPSVFIFPPKIKDVLMISLSPIVTCVVVDVSEDDPDVQISWFVNNVEVHTAQTQTHREDYNSTLRVVSALPIQHQDWMSGKEFKCKVNNKDLPAPIERTISKPKGSVRAPQVYVLPPPEEEMTKKQVTLTCMVTDFMPEDIYVEWTNNGKTELNYKNTEPVLDSDGSYFMYSKLRVEKKNWVERNSYSCSVVHEGLHNHHTTKSFSRTPGK

SEQ ID NO: 123 - protein, 19 aa, Artificial Sequence
  anti-ID B-1 HC signal sequence
MGWSWIFLFLLSGTAGVLS

SEQ ID NO: 124 - protein, 107 aa, Artificial Sequence
  anti-ID B-1 CL
RADAAPTVSIFPPSSEQLTSGGASVVCFLNNFYPKDINVKWKIDGSERQNGVLNSWTDQDSKDSTYSMSSTLTLTKDEYERHNSYTCEATHKTSTSPIVKSFNRNEC

SEQ ID NO: 125 - protein, 213 aa, Artificial Sequence
  anti-ID B-1 light chain
QIVLTQSPALMSASPGEKVTMTCSASSGVIYMYWYQQKPRSSPKPWIYLTSNLASGVPARFSGSGSGTSYSLTISSMEAEDAATYYCQQWSSNPLTFGAGTKLELKRADAAPTVSIFPPSSEQLTSGGASVVCFLNNFYPKDINVKWKIDGSERQNGVLNSWTDQDSKDSTYSMSSTLTLTKDEYERHNSYTCEATHKTSTSPIVKSFNRNEC

SEQ ID NO: 126 - protein, 22 aa, Artificial Sequence
  anti-ID B-1 LC signal sequence
MDFQVQIFSFLLMSASVIMSRG

SEQ ID NO: 127 - protein, 324 aa, Artificial Sequence; identical to SEQ ID NO: 115
  anti-ID B-2 CH

SEQ ID NO: 128 - protein, 439 aa, Artificial Sequence
  anti-ID B-2 heavy chain
QVQLQQPGAELVRPGASVKLSCKTSGYSFTRYWMNWVKQRPGQGLEWIGMIHPSDSETRLNQKFKDKATLTVDNSSSTAYMQLSSPTSEDSAVYYCASIYYEEAWGQGTLVTVSAAKTTPPSVYPLAPGSAAQTNSMVTLGCLVKGYFPEPVTVTWNSGSLSSGVHTFPAVLQSDLYTLSSSVTVPSSTWPSETVTCNVAHPASSTKVDKKIVPRDCGCKPCICTVPEVSSVFIFPPKPKDVLTITLTPKVTCVVVDISKDDPEVQFSWFVDDVEVHTAQTQPREEQFNSTFRSVSELPIMHQDWLNGKEFKCRVNSAAFPAPIEKTISKTKGRPKAPQVYTIPPPKEQMAKDKVSLTCMITDFFPEDITVEWQWNGQPAENYKNTQPIMDTDGSYFVYSKLNVQKSNWEAGNTFTCSVLHEGLHNHHTEKSLSHSPGK

SEQ ID NO: 129 - protein, 19 aa, Artificial Sequence
  anti-ID B-2 HC signal sequence
MGWSSIILFLVATATGVHS

SEQ ID NO: 130 - protein, 107 aa, Artificial Sequence; identical to SEQ ID NO: 99
  anti-ID B-2 VL

SEQ ID NO: 131 - protein, 214 aa, Artificial Sequence
  anti-ID B-2 light chain
DIQMTQSPASLSASVGETVTITCRASGNIHNYLAWYQQKQGKSPQLLVYNAKTLADSVPSRFSGSGSGTQYSLKINSLQPEDFGSYYCQHFWSTPYTFGGGTKLEIKRADAAPTVSIFPPSSEQLTSGGASVVCFLNNFYPKDINVKWKIDGSERQNGVLNSWTDQDSKDSTYSMSSTLTLTKDEYERHNSYTCEATHKTSTSPIVKSFNRNEC

SEQ ID NO: 132 - protein, 20 aa, Artificial Sequence
  anti-ID B-2 LC signal sequence
MSVLTQVLALLLLWLTGARC

SEQ ID NO: 133 - protein, 12 aa, Artificial Sequence
  spacer (IgG4hinge)
ESKYGPPCPPCP

SEQ ID NO: 134 - DNA, 36 bp, Artificial Sequence
  spacer (IgG4hinge)
gaatctaagtacggaccgccctgccccccttgccct

SEQ ID NO: 135 - protein, 119 aa, Artificial Sequence
  Hinge-CH3 spacer
ESKYGPPCPPCPGQPREPQVYTLPPSQEEMTKNQVSLTCLVKGFYPSDIAVEWESNGQPENNYKTTPPVLDSDGSFFLYSRLTVDKSRWQEGNVFSCSVMHEALHNHYTQKSLSLSLGK

SEQ ID NO: 136 - protein, 229 aa, Artificial Sequence
  Hinge-CH2-CH3 spacer
ESKYGPPCPPCPAPEFLGGPSVFLFPPKPKDTLMISRTPEVTCVVVDVSQEDPEVQFNWYVDGVEVHNAKTKPREEQFNSTYRVVSVLTVLHQDWLNGKEYKCKVSNKGLPSSIEKTISKAKGQPREPQVYTLPPSQEEMTKNQVSLTCLVKGFYPSDIAVEWESNGQPENNYKTTPPVLDSDGSFFLYSRLTVDKSRWQEGNVFSCSVMHEALHNHYTQKSLSLSLGK

SEQ ID NO: 137 - protein, 282 aa, Artificial Sequence
  IgD-hinge-Fc
RWPESPKAQASSVPTAQPQAEGSLAKATTAPATTRNTGRGGEEKKKEKEKEEQEERETKTPECPSHTQPLGVYLLTPAVQDLWLRDKATFTCFVVGSDLKDAHLTWEVAGKVPTGGVEEGLLERHSNGSQSQHSRLTLPRSLWNAGTSVTCTLNHPSLPPQRLMALREPAAQAPVKLSLNLLASSDPPEAASWLLCEVSGFSPPNILLMWLEDQREVNTSGFAPARPPPQPGSTTFWAWSVLRVPAPPSPQPATYTCVVSHEDSRTLLNASRSLEVSYVTDH

SEQ ID NO: 138 - protein, 27 aa, Artificial Sequence
  CD28 (amino acids 153-179 of Accession No. P10747)
FWVLVVVGGVLACYSLLVTVAFIIFWV

SEQ ID NO: 139 - protein, 66 aa, Artificial Sequence
  CD28 (amino acids 114-179 of Accession No. P10747)
IEVMYPPPYLDNEKSNGTIIHVKGKHLCPSPLFPGPSKPFWVLVVVGGVLACYSLLVTVAFIIFWV

SEQ ID NO: 140 - protein, 41 aa, Artificial Sequence
  CD28 (amino acids 180-220 of P10747)
RSKRSRLLHSDYMNMTPRRPGPTRKHYQPYAPPRDFAAYRS

SEQ ID NO: 141 - protein, 41 aa, Artificial Sequence
  CD28 (LL to GG)
RSKRSRGGHSDYMNMTPRRPGPTRKHYQPYAPPRDFAAYRS

SEQ ID NO: 142 - protein, 42 aa, Artificial Sequence
  4-1BB (amino acids 214-255 of Q07011.1)
KRGRKKLLYIFKQPFMRPVQTTQEEDGCSCRFPEEEEGGCEL

SEQ ID NO: 143 - protein, 112 aa, Artificial Sequence
  CD3 zeta
RVKFSRSADAPAYQQGQNQLYNELNLGRREEYDVLDKRRGRDPEMGGKPRRKNPQEGLYNELQKDKMAEAYSEIGMKGERRRGKGHDGLYQGLSTATKDTYDALHMQALPPR

SEQ ID NO: 144 - protein, 112 aa, Artificial Sequence
  CD3 zeta
RVKFSRSAEPPAYQQGQNQLYNELNLGRREEYDVLDKRRGRDPEMGGKPRRKNPQEGLYNELQKDKMAEAYSEIGMKGERRRGKGHDGLYQGLSTATKDTYDALHMQALPPR

SEQ ID NO: 145 - protein, 112 aa, Artificial Sequence
  CD3 zeta
RVKFSRSADAPAYKQGQNQLYNELNLGRREEYDVLDKRRGRDPEMGGKPRRKNPQEGLYNELQKDKMAEAYSEIGMKGERRRGKGHDGLYQGLSTATKDTYDALHMQALPPR

SEQ ID NO: 146 - protein, 24 aa, Artificial Sequence
  T2A  artificial
LEGGGEGRGSLLTCGDVEENPGPR

SEQ ID NO: 147 - protein, 357 aa, Artificial Sequence
  tEGFR  artificial
MLLLVTSLLLCELPHPAFLLIPRKVCNGIGIGEFKDSLSINATNIKHFKNCTSISGDLHILPVAFRGDSFTHTPPLDPQELDILKTVKEITGFLLIQAWPENRTDLHAFENLEIIRGRTKQHGQFSLAVVSLNITSLGLRSLKEISDGDVIISGNKNLCYANTINWKKLFGTSGQKTKIISNRGENSCKATGQVCHALCSPEGCWGPEPRDCVSCRNVSRGRECVDKCNLLEGEPREFVENSECIQCHPECLPQAMNITCTGRGPDNCIQCAHYIDGPHCVKTCPAGVMGENNTLVWKYADAGHVCHLCHPNCTYGCTGPGLEGCPTNGPKIPSIATGMVGALLLLLVVALGIGLFM

SEQ ID NO: 148 - protein, 335 aa, Artificial Sequence
  tEGFR  artificial
RKVCNGIGIGEFKDSLSINATNIKHFKNCTSISGDLHILPVAFRGDSFTHTPPLDPQELDILKTVKEITGFLLIQAWPENRTDLHAFENLEIIRGRTKQHGQFSLAVVSLNITSLGLRSLKEISDGDVIISGNKNLCYANTINWKKLFGTSGQKTKIISNRGENSCKATGQVCHALCSPEGCWGPEPRDCVSCRNVSRGRECVDKCNLLEGEPREFVENSECIQCHPECLPQAMNITCTGRGPDNCIQCAHYIDGPHCVKTCPAGVMGENNTLVWKYADAGHVCHLCHPNCTYGCTGPGLEGCPTNGPKIPSIATGMVGALLLLLVVALGIGLFM

SEQ ID NO: 149 - protein, 18 aa, Artificial Sequence
  T2A  artificial
EGRGSLLTCGDVEENPGP

SEQ ID NO: 150 - protein, 6 aa, Artificial Sequence
  MMP cleavable linker
PLGLWA

SEQ ID NO: 151 - protein, 22 aa, Artificial Sequence
  P2A
GSGATNFSLLKQAGDVEENPGP

SEQ ID NO: 152 - protein, 19 aa, Artificial Sequence
  P2A
ATNFSLLKQAGDVEENPGP

SEQ ID NO: 153 - protein, 20 aa, Artificial Sequence
  E2A
QCTNYALLKLAGDVESNPGP

SEQ ID NO: 154 - protein, 22 aa, Artificial Sequence
  F2A
VKQTLNFDLLKLAGDVESNPGP